European Patent Application EP 4 545 557 A1, published April 30, 2025. Title: SynNotch受体及其用途. Applicant: 上海恩凯细胞技术有限公司. Application CN 2023100935770, filed January 31, 2023. The sequence listing filed with the application follows.

SEQUENCE LISTING (16 sequences)

SEQ ID NO: 1 - protein, 333 aa, synthetic construct
ILDYGFIGGLGKNITPPDNEEICENEQCAELADNKICNANCNNHACGWDGGDCSLNFNDPWKNCTQSLQCWKYFNDGKCDSQCNNSGCLYDGFDCQKVEVQCNPLYDQYCRDHFQDGHCDQGCNNAECEWDGLDCDNMPENLAEGTLLIVVLMPPEKLKNNSVNFLRELSRVLHTNVVFKKDSKGEYKIYPYYGNEEELKKHHIKKRSAASWSDAPTAIFSTMKESVLPGRRRRELDQMEVRGSIVYLEIDNRQCYKSSSQCFTSATDVAAFLGALATHGNLNIPYKIEAVKSEIVETAKPPPPLYAMFSMLVIPLLIIFVIMVVIVNKKRRR

SEQ ID NO: 2 - protein, 211 aa, synthetic construct
MKLLSSIEQACDICRLKKLKCSKEKPKCAKCLKNNWECRYSPKTKRSPLTRAHLTEVESRLERLEQLFLLIFPREDLDMILKMDSLQDIKALLTGLFVQDNVNKDAVTDRLASVETDMPLTLRQHRISATSSSEESSNKGQRQLTVSAAAGGSGGSGGSDALDDFDLDMLGSDALDDFDLDMLGSDALDDFDLDMLGSDALDDFDLDMLGS

SEQ ID NO: 3 - protein, 591 aa, synthetic construct
VVSPCASRPCYNGGTCQFSPEEPFFQCFCPTNFNGLFCHILDYGFIGGLGKNITPPDNEEICENEQCAELADNKICNANCNNHACGWDGGDCSLNFNDPWKNCTQSLQCWKYFNDGKCDSQCNNSGCLYDGFDCQKVEVQCNPLYDQYCRDHFQDGHCDQGCNNAECEWDGLDCDNMPENLAEGTLLIVVLMPPEKLKNNSVNFLRELSRVLHTNVVFKKDSKGEYKIYPYYGNEEELKKHHIKKRSAASWSDAPTAIFSTMKESVLPGRRRRELDQMEVRGSIVYLEIDNRQCYKSSSQCFTSATDVAAFLGALATHGNLNIPYKIEAVKSEIVETAKPPPPLYAMFSMLVIPLLIIFVIMVVIVNKKRRREHGQLWFPMKLLSSIEQACDICRLKKLKCSKEKPKCAKCLKNNWECRYSPKTKRSPLTRAHLTEVESRLERLEQLFLLIFPREDLDMILKMDSLQDIKALLTGLFVQDNVNKDAVTDRLASVETDMPLTLRQHRISATSSSEESSNKGQRQLTVSAAAGGSGGSGGSDALDDFDLDMLGSDALDDFDLDMLGSDALDDFDLDMLGSDALDDFDLDMLGS

SEQ ID NO: 4 - protein, 750 aa, synthetic construct
MALPVTALLLPLALLLHAARPEQKLISEEDLMADVQLVESGGGLVQAGGSLRLSCAASGRTISMAAMSWFRQAPGKEREFVAGISRSAGSAVHADSVKGRFTISRDNTKNTLYLQMNSLKAEDTAVYYCAVRTSGFFGSIPRTGTAFDYWGQGTQVTVSVVSPCASRPCYNGGTCQFSPEEPFFQCFCPTNFNGLFCHILDYGFIGGLGKNITPPDNEEICENEQCAELADNKICNANCNNHACGWDGGDCSLNFNDPWKNCTQSLQCWKYFNDGKCDSQCNNSGCLYDGFDCQKVEVQCNPLYDQYCRDHFQDGHCDQGCNNAECEWDGLDCDNMPENLAEGTLLIVVLMPPEKLKNNSVNFLRELSRVLHTNVVFKKDSKGEYKIYPYYGNEEELKKHHIKKRSAASWSDAPTAIFSTMKESVLPGRRRRELDQMEVRGSIVYLEIDNRQCYKSSSQCFTSATDVAAFLGALATHGNLNIPYKIEAVKSEIVETAKPPPPLYAMFSMLVIPLLIIFVIMVVIVNKKRRREHGQLWFPMKLLSSIEQACDICRLKKLKCSKEKPKCAKCLKNNWECRYSPKTKRSPLTRAHLTEVESRLERLEQLFLLIFPREDLDMILKMDSLQDIKALLTGLFVQDNVNKDAVTDRLASVETDMPLTLRQHRISATSSSEESSNKGQRQLTVSAAAGGSGGSGGSDALDDFDLDMLGSDALDDFDLDMLGSDALDDFDLDMLGSDALDDFDLDMLGS

SEQ ID NO: 5 - DNA, 2253 bp, synthetic construct
  source 1..2253: mol_type = other DNA
atggcattgcccgtgaccgccctgctgctgccactggccttgttgctccacgccgcgcggccagaacagaagctgatcagcgaggaggatctgatggctgatgtgcaactcgtagagtccggtggcggactcgtccaggcgggaggctccctgcgcctgagttgcgctgcgtccggaagaactattagcatggccgccatgagttggttcagacaggcgcctggaaaggagagggagttcgtggcaggcataagtcgctccgcagggtcagccgtccatgccgactccgtaaagggacgctttaccatctccagagataacacaaaaaacacgctctatctccaaatgaattctttgaaggccgaggacacagccgtgtactactgcgccgttaggaccagcggattttttggaagcattcctaggacagggacagcctttgattactggggccagggaacgcaggttaccgtttccgtcgtcagcccgtgcgcgtcccgcccttgttacaacggagggacctgccaattctcccccgaggaacctttcttccagtgcttctgccccacgaacttcaacggcctcttctgccacatcttggattacggcttcatcggaggcctgggcaagaacatcacccctcccgacaatgaggaaatctgcgagaatgagcagtgcgccgagctggccgacaacaagatctgcaacgccaactgcaacaaccacgcctgcgggtgggacggcggcgactgctctctcaacttcaacgacccctggaagaactgcacccagtcgctgcagtgctggaaatacttcaacgacggcaaatgcgactcgcagtgcaacaactccggctgcctgtacgacggcttcgactgccagaaagtggaggttcagtgcaaccctttgtacgaccagtattgcagggatcactttcaagacggccattgcgaccaaggctgtaacaacgcagagtgcgaatgggacggcctggactgtgacaacatgccggagaacctggccgaaggcaccctgttgatagtcgtcctgatgccccccgaaaagctgaagaacaactccgtcaacttcctccgagagctgagccgagtgctccacaccaacgtggtgttcaagaaagacagcaaaggcgaatacaagatctacccttactatggcaacgaggaggagctgaagaaacatcacatcaagaagaggtcggcggcttcctggtcggatgctcctaccgccatcttcagtaccatgaaggagtccgtcttaccaggaaggcgccgtagggagttggaccaaatggaagtcagggggtcaatcgtatacttagaaatagacaaccgccagtgctacaaatcctcctcccagtgcttcaccagcgccaccgacgtggccgccttcctcggggctttggccacccatggcaatctgaacatcccctataagatcgaggctgtgaaaagtgagatagtcgagaccgccaagccgccgccgccgctttatgccatgttttccatgttggtcatcccgttgctgatcatcttcgtcatcatggtggtcatcgtgaataagaagcggcgccgcgaacacgggcagctgtggttccccatgaagctgctgagcagcatcgagcaggcctgtgacatctgccggctgaagaaactgaagtgcagcaaagaaaagcccaagtgcgccaagtgcctgaagaacaactgggagtgccggtacagccccaagaccaagagaagccccctgaccagagcccacctgaccgaggtggaaagccggctggaaagactggaacagctgtttctgctgatcttcccacgcgaggacctggacatgatcctgaagatggacagcctgcaggacatcaaggccctgctgaccggcctgttcgtgcaggacaacgtgaacaaggacgccgtgaccgacagactggccagcgtggaaaccgacatgcccctgaccctgcggcagcacagaatcagcgccaccagcagcagcgaggaaagcagcaacaagggccagcggcagctgacagtgtctgctgctgcaggcggaagcggaggctctggcggatctgatgccctggacgacttcgacctggatatgctgggcagcgacgccctggatgattttgatctggacatgctgggatctgacgctctggacgatttcgatctcgacatgttgggatcagatgcactggatgactttgacctggacatgctcggatcatga

SEQ ID NO: 6 - protein, 696 aa, synthetic construct
MALPVTALLLPLALLLHAARPEQKLISEEDLMADVQLVESGGGLVQAGGSLRLSCAASGRTISMAAMSWFRQAPGKEREFVAGISRSAGSAVHADSVKGRFTISRDNTKNTLYLQMNSLKAEDTAVYYCAVRTSGFFGSIPRTGTAFDYWGQGTQVTVSILDYSFTGGAGRDIPPPQIEEACELPECQVDAGNKVCNLQCNNHACGWDGGDCSLNFNDPWKNCTQSLQCWKYFSDGHCDSQCNSAGCLFDGFDCQLTEGQCNPLYDQYCKDHFSDGHCDQGCNSAECEWDGLDCAEHVPERLAAGTLVLVVLLPPDQLRNNSFHFLRELSHVLHTNVVFKRDAQGQQMIFPYYGHEEELRKHPIKRSTVGWATSSLLPGTSGGRQRRELDPMDIRGSIVYLEIDNRQCVQSSSQCFQSATDVAAFLGALASLGSLNIPYKIEAVKSEPVEPPLPSQLHLMYVAAAAFVLLFFVGCGVLLSRKRRRMKLLSSIEQACDICRLKKLKCSKEKPKCAKCLKNNWECRYSPKTKRSPLTRAHLTEVESRLERLEQLFLLIFPREDLDMILKMDSLQDIKALLTGLFVQDNVNKDAVTDRLASVETDMPLTLRQHRISATSSSEESSNKGQRQLTVSAAAGGSGGSGGSDALDDFDLDMLGSDALDDFDLDMLGSDALDDFDLDMLGSDALDDFDLDMLGS

SEQ ID NO: 7 - DNA, 2091 bp, synthetic construct
  source 1..2091: mol_type = other DNA
atggcattgcccgtgaccgccctgctgctgccactggccttgttgctccacgccgcgcggccagaacagaagctgatcagcgaggaggatctgatggctgatgtgcaactcgtagagtccggtggcggactcgtccaggcgggaggctccctgcgcctgagttgcgctgcgtccggaagaactattagcatggccgccatgagttggttcagacaggcgcctggaaaggagagggagttcgtggcaggcataagtcgctccgcagggtcagccgtccatgccgactccgtaaagggacgctttaccatctccagagataacacaaaaaacacgctctatctccaaatgaattctttgaaggccgaggacacagccgtgtactactgcgccgttaggaccagcggattttttggaagcattcctaggacagggacagcctttgattactggggccagggaacgcaggttaccgtttccatcctggactacagcttcacaggtggcgctgggcgcgacattcccccaccgcagattgaggaggcctgtgagctgcctgagtgccaggtggatgcaggcaataaggtctgcaacctgcagtgtaataatcacgcatgtggctgggatggtggcgactgctccctcaacttcaatgacccctggaagaactgcacgcagtctctacagtgctggaagtattttagcgacggccactgtgacagccagtgcaactcggccggctgcctctttgatggcttcgactgccagctcaccgagggacagtgcaaccccctgtatgaccagtactgcaaggaccacttcagtgatggccactgcgaccagggctgtaacagtgccgaatgtgagtgggatggcctagactgtgctgagcatgtacccgagcggctggcagccggcaccctggtgctggtggtgctgcttccacccgaccagctacggaacaactccttccactttctgcgggagctcagccacgtgctgcacaccaacgtggtcttcaagcgtgatgcgcaaggccagcagatgatcttcccgtactatggccacgaggaagagctgcgcaagcacccaatcaagcgctctacagtgggttgggccacctcttcactgcttcctggtaccagtggtgggcgccagcgcagggagctggaccccatggacatccgtggctccattgtctacctggagatcgacaaccggcaatgtgtgcagtcatcctcgcagtgcttccagagtgccaccgatgtggctgccttcctaggtgctcttgcgtcacttggcagcctcaatattccttacaagattgaggccgtgaagagtgagccggtggagcctccgctgccctcgcagctgcacctcatgtacgtggcagcggccgccttcgtgctcctgttctttgtgggctgtggggtgctgctgtcccgcaagcgccggcggatgaagctgctgagcagcatcgagcaggcctgtgacatctgccggctgaagaaactgaagtgcagcaaagaaaagcccaagtgcgccaagtgcctgaagaacaactgggagtgccggtacagccccaagaccaagagaagccccctgaccagagcccacctgaccgaggtggaaagccggctggaaagactggaacagctgtttctgctgatcttcccacgcgaggacctggacatgatcctgaagatggacagcctgcaggacatcaaggccctgctgaccggcctgttcgtgcaggacaacgtgaacaaggacgccgtgaccgacagactggccagcgtggaaaccgacatgcccctgaccctgcggcagcacagaatcagcgccaccagcagcagcgaggaaagcagcaacaagggccagcggcagctgacagtgtctgctgctgcaggcggaagcggaggctctggcggatctgatgccctggacgacttcgacctggatatgctgggcagcgacgccctggatgattttgatctggacatgctgggatctgacgctctggacgatttcgatctcgacatgttgggatcagatgcactggatgactttgacctggacatgctcggatcatga

SEQ ID NO: 8 - protein, 310 aa, synthetic construct
METDTLLLWVLLLWVPGSTGDMVSKGEELFTGVVPILVELDGDVNGHKFSVSGEGEGDATYGKLTLKFICTTGKLPVPWPTLVTTLTYGVQCFSRYPDHMKQHDFFKSAMPEGYVQERTIFFKDDGNYKTRAEVKFEGDTLVNRIELKGIDFKEDGNILGHKLEYNYNSHNVYIMADKQKNGIKVNFKIRHNIEDGSVQLADHYQQNTPIGDGPVLLPDNHYLSTQSALSKDPNEKRDHMVLLEFVTAAGITLGMDELYKNAVGQDTQEVIVVPHSLPFKVVVISAILALVVLTIISLIILIMLWQKKPR

SEQ ID NO: 9 - DNA, 930 bp, synthetic construct
  source 1..930: mol_type = other DNA
atggagaccgacaccctgctgctgtgggtgctgctgctgtgggtgcccggcagcaccggcgacatggtgagcaagggcgaggagctgttcaccggcgtggtgcccatcctggtggagctggacggcgacgtgaacggccacaagttcagcgtgagcggcgagggcgagggcgacgccacctacggcaagctgaccctgaagttcatctgcaccaccggcaagctgcccgtgccctggcccaccctggtgaccaccctgacctacggcgtgcagtgcttcagccgctaccccgaccacatgaagcagcacgacttcttcaagagcgccatgcccgagggctacgtgcaggagcgcaccatcttcttcaaggacgacggcaactacaagacccgcgccgaggtgaagttcgagggcgacaccctggtgaaccgcatcgagctgaagggcatcgacttcaaggaggacggcaacatcctgggccacaagctggagtacaactacaacagccacaacgtgtacatcatggccgacaagcagaagaacggcatcaaggtgaacttcaagatccgccacaacatcgaggacggcagcgtgcagctggccgaccactaccagcagaacacccccatcggcgacggccccgtgctgctgcccgacaaccactacctgagcacccagagcgccctgagcaaggaccccaacgagaagcgcgaccacatggtgctgctggagttcgtgaccgccgccggcatcaccctgggcatggacgagctgtacaagaacgccgtgggccaggacacccaggaggtgatcgtggtgccccacagcctgcccttcaaggtggtggtgatcagcgccatcctggccctggtggtgctgaccatcatcagcctgatcatcctgatcatgctgtggcagaagaagccccgc

SEQ ID NO: 10 - protein, 496 aa, synthetic construct
MALPVTALLLPLALLLHAARPEQKLISEEDLDIQMTQTTSSLSASLGDRVTISCRASQDISKYLNWYQQKPDGTVKLLIYHTSRLHSGVPSRFSGSGSGTDYSLTISNLEQEDIATYFCQQGNTLPYTFGGGTKLEITGGGGSGGGGSGGGGSEVKLQESGPGLVAPSQSLSVTCTVSGVSLPDYGVSWIRQPPRKGLEWLGVIWGSETTYYNSALKSRLTIIKDNSKSQVFLKMNSLQTDDTAIYYCAKHYYYGGSYAMDYWGQGTSVTVSSKPTTTPAPRPPTPAPTIASQPLSLRPEACRPAAGGAVHTRGLDFACDIYIWAPLAGTCGVLLLSLVITKRGRKKLLYIFKQPFMRPVQTTQEEDGCSCRFPEEEEGGCELRVKFSRSADAPAYQQGQNQLYNELNLGRREEYDVLDKRRGRDPEMGGKPQRRKNPQEGLYNELQKDKMAEAYSEIGMKGERRRGKGHDGLYQGLSTATKDTYDALHMQALPPR

SEQ ID NO: 11 - DNA, 1759 bp, synthetic construct
  source 1..1759: mol_type = other DNA
ggagcactgtcctccgaacgtcggagcactgtcctccgaacgtcggagcactgtcctccgaacgtcggagcactgtcctccgaacggagcatgtcctccgaacgtcggagcactgtcctccgaacgactagttaggcgtgtacggtgggaggcctatataagcagagctcgtttagtgaaccgtcagatcgcctggagacgccatccacgctgttttgacctccatagaagacaccgggaccgatccagcctctcgacattcgttggatccatggcattgcccgtgaccgccctgctgctgccactggccttgttgctccacgccgcgcggccagaacagaagctgatcagcgaggaggatctggatatacagatgacgcagacaacgtcaagtctttccgccagcttgggagaccgagtgactatatcttgtagagcaagccaggatatttctaagtatcttaactggtaccaacaaaagcccgatggaacggttaagctgcttatataccataccagtagactccactccggcgtaccatcacggttttctggcagtggctccgggaccgactattctttgacgatctctaatctcgaacaagaggatattgcaacatacttttgtcagcaaggcaataccttgccatatacgtttgggggcgggacaaaacttgagataaccggcggcggtggttcaggcggtggcggttccggtggtgggggatcagaggttaagcttcaggaatccggaccaggtttggttgcccccagccaatctctcagcgttacatgcacggtttcaggcgtcagtctccccgattacggtgtaagttggattcggcaacctccgcgaaagggtctggaatggctgggggttatttgggggagtgagacaacttattacaactctgcacttaagagtcggcttaccatcatcaaggataattcaaaatcacaagtattcctgaagatgaactcattgcaaacagatgatacagctatatactattgtgccaagcattactattatggtggttcttatgcaatggattactgggggcaaggcacgtcagtgacagtgagttcaaagcccaccacgacgccagcgccgcgaccaccaacaccggcgcccaccatcgcgtcgcagcccctgtccctgcgcccagaggcgtgccggccagcggcggggggcgcagtgcacacgagggggctggacttcgcctgtgatatctacatctgggcgcccttggccgggacttgtggggtccttctcctgtcactggttatcaccaaacggggcagaaagaaactcctgtatatattcaaacaaccatttatgagaccagtacaaactactcaagaggaagatggctgtagctgccgatttccagaagaagaagaaggaggatgtgaactgagagtgaagttcagcaggagcgcagacgcccccgcgtaccagcagggccagaaccagctctataacgagctcaatctaggacgaagagaggagtacgatgttttggacaagagacgtggccgggaccctgagatggggggaaagccgcagagaaggaagaaccctcaggaaggcctgtacaatgaactgcagaaagataagatggcggaggcctacagtgagattgggatgaaaggcgagcgccggaggggcaaggggcacgatggcctttaccagggtctcagtacagccaccaaggacacctacgacgcccttcacatgcaggccctgccccctcgc

SEQ ID NO: 12 - protein, 370 aa, synthetic construct
METDTLLLWVLLLWVPGSTGDYPYDVPDYAGAQPARPEEPLVVKVEEGDNAVLQCLKGTSDGPTQQLTWSRESPLKPFLKLSLGLPGLGIHMRPLAIWLFIFNVSQQMGGFYLCQPGPPSEKAWQPGWTVNVEGSGELFRWNVSDLGGLGCGLKNRSSEGPSSPSGKLMSPKLYVWAKDRPEIWEGEPPCLPPRDSLNQSLSQDLTMAPGSTLWLSCGVPPDSVSRGPLSWTHVHPKGPKSLLSLELKDDRPARDMWVMETGLLLPRATAQDAGKYYCHRGNLTMSFHLEITARPVLWHWLLRTGGWKVDEQKLISEEDLNAVGQDTQEVIVVPHSLPFKVVVISAILALVVLTIISLIILIMLWQKKPR

SEQ ID NO: 13 - DNA, 1110 bp, synthetic construct
  source 1..1110: mol_type = other DNA
atggagaccgacaccctgctgctgtgggtgctgctgctgtgggtgcccggcagcaccggcgactacccctacgacgtgcccgactacgccggcgcccagcccgcccgccccgaggagcccctggtggtgaaggtggaggagggcgacaacgccgtgctgcagtgcctgaagggcaccagcgacggccccacccagcagctgacctggagccgcgagagccccctgaagcccttcctgaagctgagcctgggcctgcccggcctgggcatccacatgcgccccctggccatctggctgttcatcttcaacgtgagccagcagatgggcggcttctacctgtgccagcccggcccccccagcgagaaggcctggcagcccggctggaccgtgaacgtggagggcagcggcgagctgttccgctggaacgtgagcgacctgggcggcctgggctgcggcctgaagaaccgcagcagcgagggccccagcagccccagcggcaagctgatgagccccaagctgtacgtgtgggccaaggaccgccccgagatctgggagggcgagcccccctgcctgcccccccgcgacagcctgaaccagagcctgagccaggacctgaccatggcccccggcagcaccctgtggctgagctgcggcgtgccccccgacagcgtgagccgcggccccctgagctggacccacgtgcaccccaagggccccaagagcctgctgagcctggagctgaaggacgaccgccccgcccgcgacatgtgggtgatggagaccggcctgctgctgccccgcgccaccgcccaggacgccggcaagtactactgccaccgcggcaacctgaccatgagcttccacctggagatcaccgcccgccccgtgctgtggcactggctgctgcgcaccggcggctggaaggtggacgagcagaagctgatcagcgaggaggacctgaacgccgtgggccaggacacccaggaggtgatcgtggtgccccacagcctgcccttcaaggtggtggtgatcagcgccatcctggccctggtggtgctgaccatcatcagcctgatcatcctgatcatgctgtggcagaagaagccccgc

SEQ ID NO: 14 - DNA, 250 bp, synthetic construct
  source 1..250: mol_type = other DNA
ggagcactgtcctccgaacgtcggagcactgtcctccgaacgtcggagcactgtcctccgaacgtcggagcactgtcctccgaacggagcatgtcctccgaacgtcggagcactgtcctccgaacgactagttaggcgtgtacggtgggaggcctatataagcagagctcgtttagtgaaccgtcagatcgcctggagacgccatccacgctgttttgacctccatagaagacaccgggaccgatccagc

SEQ ID NO: 15 - protein, 39 aa, synthetic construct
VVSPCASRPCYNGGTCQFSPEEPFFQCFCPTNFNGLFCH

SEQ ID NO: 16 - protein, 8 aa, synthetic construct
EHGQLWFP